European Patent Specification EP 4 063 491 B1, published November 13, 2024. Title: COMPOSITION FOR CULTURING NATURAL KILLER CELL AND METHOD FOR PRODUCING NATURAL KILLER CELL USING THE SAME. Applicant: GI Cell, Inc. The sequence listing filed with the application follows.

SEQUENCE LISTING (46 sequences)

SEQ ID NO: 1 - protein, 25 aa, Artificial Sequence
  signal peptide (TPA)
MDAMLRGLCCVLLLCGAVFVSPSHA

SEQ ID NO: 2 - protein, 208 aa, Artificial Sequence [sequence omitted]

SEQ ID NO: 3 - protein, 30 aa, Artificial Sequence
  hinge with linker
GSGGGGSGGGGSGGGGSAESKYGPPCPPCP

SEQ ID NO: 4 - protein, 216 aa, Artificial Sequence
  immunoglobulin fc
APEAAGGPSVFLFPPKPKDQLMISRTPEVTCVVVDVSQEDPEVQFNWYVDGVEVHNAKTKPREEQFNSTYRVVSVLTVLHQDWLNGKEYKCKVSNKGLPSSIEKTISKAKGQPREPQVYTLPPSQEEMTKNQVSLTCLVKGFYPSDIAVEWESNGQPENNYKTTPPVLDSDGSFFLYSRLTVDKSRWQEGNVFSCSVLHEALHNHYTQKSLSLSLG

SEQ ID NO: 5 - protein, 5 aa, Artificial Sequence
  linker
GGGGS

SEQ ID NO: 6 - protein, 133 aa, Artificial Sequence
  hIL-2M
APTSSSTKKTQLQLEHLLLDLQMILNGINNYKNPKLTAMLTAKFYMPKKATELKHLQCLEEELKPLEEVLNLAQSKNFHLRPRDLISNINVIVLELKGSETTFMCEYADETATIVEFLNRWITFCQSIISTLT

SEQ ID NO: 7 - protein, 617 aa, Artificial Sequence
  fusion protein comprising variants of IL-2 and fragments of CD80
MDAMLRGLCCVLLLCGAVFVSPSHAVIHVTKEVKEVATLSCGHNVSVEELAQTRIYWQKEKKMVLTMMSGDMNIWPEYKNRTIFDITNNLSIVILALRPSDEGTYECVVLKYEKDAFKREHLAEVTLSVKADFPTPSISDFEIPTSNIRRIICSTSGGFPEPHLSWLENGEELNAINTTVSQDPETELYAVSSKLDFNMTTNHSFMCLIKYGHLRVNQTFNWNTTKQEHFPDNGSGGGGSGGGGSGGGGSAESKYGPPCPPCPAPEAAGGPSVFLFPPKPKDQLMISRTPEVTCVVVDVSQEDPEVQFNWYVDGVEVHNAKTKPREEQFNSTYRVVSVLTVLHQDWLNGKEYKCKVSNKGLPSSIEKTISKAKGQPREPQVYTLPPSQEEMTKNQVSLTCLVKGFYPSDIAVEWESNGQPENNYKTTPPVLDSDGSFFLYSRLTVDKSRWQEGNVFSCSVLHEALHNHYTQKSLSLSLGGGGGSAPTSSSTKKTQLQLEHLLLDLQMILNGINNYKNPKLTAMLTAKFYMPKKATELKHLQCLEEELKPLEEVLNLAQSKNFHLRPRDLISNINVIVLELKGSETTFMCEYADETATIVEFLNRWITFCQSIISTLT

SEQ ID NO: 8 - DNA, 1857 bp, Artificial Sequence
  nucleotiedes coding fusion protein (GI101)
atggatgctatgctgagaggcctgtgttgcgtgctgctgctgtgtggcgctgtgttcgtgtctccttctcacgctgtgatccacgtgaccaaagaagtgaaagaggtcgccacactgtcctgcggccacaacgtttcagtggaagaactggcccagaccaggatctactggcagaaagaaaagaaaatggtgctgaccatgatgtccggcgacatgaacatctggcctgagtacaagaaccggaccatcttcgacatcaccaacaacctgtccatcgtgattctggccctgaggccttctgatgagggcacctatgagtgcgtggtgctgaagtacgagaaggacgccttcaagcgcgagcacctggctgaagtgacactgtccgtgaaggccgactttcccacaccttccatctccgacttcgagatccctacctccaacatccggcggatcatctgttctacctctggcggctttcctgagcctcacctgtcttggctggaaaacggcgaggaactgaacgccatcaacaccaccgtgtctcaggaccccgaaaccgagctgtacgctgtgtcctccaagctggacttcaacatgaccaccaaccacagcttcatgtgcctgattaagtacggccacctgagagtgaaccagaccttcaactggaacaccaccaagcaagagcacttccctgacaatggatctggcggcggaggttctggcggaggtggaagcggaggcggaggatctgctgagtctaagtatggccctccttgtcctccatgtcctgctccagaagctgctggcggaccctctgtgttcctgtttcctccaaagcctaaggaccagctcatgatctctcggacacccgaagtgacctgcgtggtggtggatgtgtctcaagaggaccctgaggtgcagttcaattggtacgtggacggcgtggaagtgcacaacgccaagaccaagcctagagaggaacagttcaactccacctacagagtggtgtccgtgctgaccgtgctgcaccaggattggctgaacggcaaagagtacaagtgcaaggtgtccaacaagggcctgccttccagcatcgaaaagaccatctccaaggctaagggccagcctagggaaccccaggtttacaccctgcctccaagccaagaggaaatgaccaagaaccaggtgtccctgacctgcctggtcaagggcttctacccttccgacattgccgtggaatgggagtccaatggccagcctgagaacaactacaagaccacacctcctgtgctggactccgacggctccttctttctgtactctcgcctgaccgtggacaagtctagatggcaagagggcaacgtgttctcctgctctgtgctgcacgaggccctgcacaatcactacacccagaagtccctgtctctgtctcttggaggtggtggcggttctgcccctaccagctcctctaccaagaaaacccagctccagttggagcatctgctgctggacctccagatgattctgaacgggatcaacaactataagaaccccaagctgaccgccatgctgaccgctaagttctacatgcccaagaaggccaccgagctgaagcacctccagtgcctggaagaagaactgaagcccctggaagaggtgctgaatctggcccagtccaagaacttccacctgaggccacgggacctgatcagcaacatcaacgtgatcgtgctggaactgaagggctccgagacaacctttatgtgcgagtacgccgacgagacagccaccatcgtggaatttctgaaccggtggatcaccttctgccagagcatcatctccacactgacctgatga

SEQ ID NO: 9 - protein, 592 aa, Artificial Sequence
  fusion protein (GI101)
VIHVTKEVKEVATLSCGHNVSVEELAQTRIYWQKEKKMVLTMMSGDMNIWPEYKNRTIFDITNNLSIVILALRPSDEGTYECVVLKYEKDAFKREHLAEVTLSVKADFPTPSISDFEIPTSNIRRIICSTSGGFPEPHLSWLENGEELNAINTTVSQDPETELYAVSSKLDFNMTTNHSFMCLIKYGHLRVNQTFNWNTTKQEHFPDNGSGGGGSGGGGSGGGGSAESKYGPPCPPCPAPEAAGGPSVFLFPPKPKDQLMISRTPEVTCVVVDVSQEDPEVQFNWYVDGVEVHNAKTKPREEQFNSTYRVVSVLTVLHQDWLNGKEYKCKVSNKGLPSSIEKTISKAKGQPREPQVYTLPPSQEEMTKNQVSLTCLVKGFYPSDIAVEWESNGQPENNYKTTPPVLDSDGSFFLYSRLTVDKSRWQEGNVFSCSVLHEALHNHYTQKSLSLSLGGGGGSAPTSSSTKKTQLQLEHLLLDLQMILNGINNYKNPKLTAMLTAKFYMPKKATELKHLQCLEEELKPLEEVLNLAQSKNFHLRPRDLISNINVIVLELKGSETTFMCEYADETATIVEFLNRWITFCQSIISTLT

SEQ ID NO: 10 - protein, 133 aa, Artificial Sequence [sequence omitted]

SEQ ID NO: 11 - protein, 288 aa, Artificial Sequence
  CD80
MGHTRRQGTSPSKCPYLNFFQLLVLAGLSHFCSGVIHVTKEVKEVATLSCGHNVSVEELAQTRIYWQKEKKMVLTMMSGDMNIWPEYKNRTIFDITNNLSIVILALRPSDEGTYECVVLKYEKDAFKREHLAEVTLSVKADFPTPSISDFEIPTSNIRRIICSTSGGFPEPHLSWLENGEELNAINTTVSQDPETELYAVSSKLDFNMTTNHSFMCLIKYGHLRVNQTFNWNTTKQEHFPDNLLPSWAITLISVNGIFVICCLTYCFAPRCRERRRNERLRRESVRPV

SEQ ID NO: 12 - protein, 215 aa, Artificial Sequence
  modified Fc
SHTQPLGVFLFPPKPKDTLMISRTPEVTCVVVDVSQEDPEVQFNWYVDGVEVHNAKTKPREEQFNSTYRVVSVLTVLHQDWLNGKEYKCKVSNKGLPSSIEKTISKAKGQPREPQVYTLPPSQEEMTKNQVSLTCLVKGFYPSDIAVEWESNGQPENNYKTTPPVLDSDGSFFLYSRLTVDKSRWQEGNVFSCSVMHEALHNHYTQKSLSLSLGK

SEQ ID NO: 13 - protein, 306 aa, Artificial Sequence
  mCD80
MACNCQLMQDTPLLKFPCPRLILLFVLLIRLSQVSSDVDEQLSKSVKDKVLLPCRYNSPHEDESEDRIYWQKHDKVVLSVIAGKLKVWPEYKNRTLYDNTTYSLIILGLVLSDRGTYSCVVQKKERGTYEVKHLALVKLSIKADFSTPNITESGNPSADTKRITCFASGGFPKPRFSWLENGRELPGINTTISQDPESELYTISSQLDFNTTRNHTIKCLIKYGDAHVSEDFTWEKPPEDPPDSKNTLVLFGAGFGAVITVVVIVVIIKCFCKHRSCFRRNEASRETNNSLTFGPEEALAEQTVFL

SEQ ID NO: 14 - DNA, 1848 bp, Artificial Sequence
  nucleotiedes coding fusion protein (mGI101)
atggatgctatgctgagaggcctgtgttgcgtgctgctgctgtgtggcgctgtgttcgtgtctccttctcacgctgtggacgagcagctctccaagtccgtgaaggataaggtcctgctgccttgccggtacaactctcctcacgaggacgagtctgaggaccggatctactggcagaaacacgacaaggtggtgctgtccgtgatcgccggaaagctgaaagtgtggcctgagtacaagaacaggaccctgtacgacaacaccacctacagcctgatcatcctgggcctcgtgctgagcgatagaggcacctattcttgcgtggtgcagaagaaagagcggggcacctacgaagtgaagcacctggctctggtcaagctgtccatcaaggccgacttcagcacccctaacatcaccgagtctggcaacccttccgccgacaccaagagaatcacctgtttcgcctctggcggcttccctaagcctcggttctcttggctggaaaacggcagagagctgcccggcatcaataccaccatttctcaggacccagagtccgagctgtacaccatctccagccagctcgactttaacaccaccagaaaccacaccatcaagtgcctgattaagtacggcgacgcccacgtgtccgaggactttacttgggagaaacctcctgaggaccctcctgactctggatctggcggcggaggttctggcggaggtggaagcggaggcggaggatctgctgagtctaagtatggccctccttgtcctccatgtcctgctccagaagctgctggcggaccctctgtgttcctgtttcctccaaagcctaaggaccagctcatgatctctcggacccctgaagtgacctgcgtggtggtggatgtgtctcaagaggaccctgaggtgcagttcaattggtacgtggacggcgtggaagtgcacaacgccaagaccaagcctagagaggaacagttcaactccacctatagagtggtgtccgtgctgaccgtgctgcaccaggattggctgaacggcaaagagtacaagtgcaaggtgtccaacaagggcctgccttccagcatcgaaaagaccatcagcaaggctaagggccagcctagggaaccccaggtttacaccctgcctccaagccaagaggaaatgaccaagaaccaggtgtccctgacctgcctggtcaagggcttctacccttccgacattgccgtggaatgggagtccaatggccagcctgagaacaactacaagaccacacctcctgtgctggactccgacggctccttctttctgtactctcgcctgaccgtggacaagtctaggtggcaagagggcaacgtgttctcctgctctgtgctgcacgaggctctgcacaaccactacacccagaagtccctgtctctgtctcttggaggtggtggcggttctgcccctacctccagctctaccaagaaaacccagctccagttggagcatctgctgctggacctccagatgatcctgaatggcatcaacaattacaagaaccccaagctgaccgccatgctgaccgctaagttctacatgcccaagaaggccaccgagctgaagcacttgcagtgcctggaagaggaactgaagcccctggaagaagtgctgaatctggcccagtccaagaacttccacctgaggcctagggacctgatctccaacatcaacgtgatcgtgctggaactgaaaggctccgagacaaccttcatgtgcgagtacgccgacgagacagccaccatcgtggaatttctgaaccggtggatcaccttctgccagagcatcatctccacactgacc

SEQ ID NO: 15 - protein, 616 aa, Artificial Sequence
  fusion protein (mGI101)
MDAMLRGLCCVLLLCGAVFVSPSHAVDEQLSKSVKDKVLLPCRYNSPHEDESEDRIYWQKHDKVVLSVIAGKLKVWPEYKNRTLYDNTTYSLIILGLVLSDRGTYSCVVQKKERGTYEVKHLALVKLSIKADFSTPNITESGNPSADTKRITCFASGGFPKPRFSWLENGRELPGINTTISQDPESELYTISSQLDFNTTRNHTIKCLIKYGDAHVSEDFTWEKPPEDPPDSGSGGGGSGGGGSGGGGSAESKYGPPCPPCPAPEAAGGPSVFLFPPKPKDQLMISRTPEVTCVVVDVSQEDPEVQFNWYVDGVEVHNAKTKPREEQFNSTYRVVSVLTVLHQDWLNGKEYKCKVSNKGLPSSIEKTISKAKGQPREPQVYTLPPSQEEMTKNQVSLTCLVKGFYPSDIAVEWESNGQPENNYKTTPPVLDSDGSFFLYSRLTVDKSRWQEGNVFSCSVLHEALHNHYTQKSLSLSLGGGGGSAPTSSSTKKTQLQLEHLLLDLQMILNGINNYKNPKLTAMLTAKFYMPKKATELKHLQCLEEELKPLEEVLNLAQSKNFHLRPRDLISNINVIVLELKGSETTFMCEYADETATIVEFLNRWITFCQSIISTLT

SEQ ID NO: 16 - DNA, 1437 bp, Artificial Sequence
  nucleotiedes coding fusion protein (GI101C1)
atggatgctatgctgagaggcctgtgttgcgtgctgctgctgtgtggcgctgtgttcgtgtctccttctcacgctgtgatccacgtgaccaaagaagtgaaagaggtcgccacactgtcctgcggccacaacgtttcagtggaagaactggcccagaccaggatctactggcagaaagaaaagaaaatggtgctgaccatgatgtccggcgacatgaacatctggcctgagtacaagaaccggaccatcttcgacatcaccaacaacctgtccatcgtgattctggccctgaggccttctgatgagggcacctatgagtgcgtggtgctgaagtacgagaaggacgccttcaagcgcgagcacctggctgaagtgacactgtccgtgaaggccgactttcccacaccttccatctccgacttcgagatccctacctccaacatccggcggatcatctgttctacctctggcggctttcctgagcctcacctgtcttggctggaaaacggcgaggaactgaacgccatcaacaccaccgtgtctcaggaccccgaaaccgagctgtacgctgtgtcctccaagctggacttcaacatgaccaccaaccacagcttcatgtgcctgattaagtacggccacctgagagtgaaccagaccttcaactggaacaccaccaagcaagagcacttccctgacaatggatctggcggcggaggttctggcggaggtggaagcggaggcggaggatctgctgagtctaagtatggccctccttgtcctccatgtcctgctccagaagctgctggcggaccctctgtgttcctgtttcctccaaagcctaaggaccagctcatgatctctcggacacccgaagtgacctgcgtggtggtggatgtgtctcaagaggaccctgaggtgcagttcaattggtacgtggacggcgtggaagtgcacaacgccaagaccaagcctagagaggaacagttcaactccacctacagagtggtgtccgtgctgaccgtgctgcaccaggattggctgaacggcaaagagtacaagtgcaaggtgtccaacaagggcctgccttccagcatcgaaaagaccatctccaaggctaagggccagcctagggaaccccaggtttacaccctgcctccaagccaagaggaaatgaccaagaaccaggtgtccctgacctgcctggtcaagggcttctacccttccgacattgccgtggaatgggagtccaatggccagcctgagaacaactacaagaccacacctcctgtgctggactccgacggctccttctttctgtactctcgcctgaccgtggacaagtctaggtggcaagagggcaacgtgttctcctgctctgtgctgcacgaggccctgcacaatcactacacccagaagtccctgtctctgtccctgggc

SEQ ID NO: 17 - protein, 454 aa, Artificial Sequence
  fusion protein (GI101C1)
VIHVTKEVKEVATLSCGHNVSVEELAQTRIYWQKEKKMVLTMMSGDMNIWPEYKNRTIFDITNNLSIVILALRPSDEGTYECVVLKYEKDAFKREHLAEVTLSVKADFPTPSISDFEIPTSNIRRIICSTSGGFPEPHLSWLENGEELNAINTTVSQDPETELYAVSSKLDFNMTTNHSFMCLIKYGHLRVNQTFNWNTTKQEHFPDNGSGGGGSGGGGSGGGGSAESKYGPPCPPCPAPEAAGGPSVFLFPPKPKDQLMISRTPEVTCVVVDVSQEDPEVQFNWYVDGVEVHNAKTKPREEQFNSTYRVVSVLTVLHQDWLNGKEYKCKVSNKGLPSSIEKTISKAKGQPREPQVYTLPPSQEEMTKNQVSLTCLVKGFYPSDIAVEWESNGQPENNYKTTPPVLDSDGSFFLYSRLTVDKSRWQEGNVFSCSVLHEALHNHYTQKSLSLSLG

SEQ ID NO: 18 - DNA, 1176 bp, Artificial Sequence
  nucleotiedes coding fusion protein (GI101C2)
atggatgctatgctgagaggcctgtgttgcgtgctgctgctgtgtggcgctgtgttcgtgtctccatctcacgccgctgagtctaagtacggccctccttgtcctccatgtcctgctccagaagctgctggcggaccctctgtgttcctgtttcctccaaagcctaaggaccagctcatgatctctcggacccctgaagtgacctgcgtggtggtggatgtgtctcaagaggaccctgaggtgcagttcaattggtacgtggacggcgtggaagtgcacaacgccaagaccaagcctagagaggaacagttcaactccacctacagagtggtgtccgtgctgaccgtgctgcaccaggattggctgaacggcaaagagtacaagtgcaaggtgtccaacaagggcctgccttccagcatcgaaaagaccatctccaaggctaagggccagcctagggaaccccaggtttacaccctgcctccaagccaagaggaaatgaccaagaaccaggtgtccctgacctgcctggtcaagggcttctacccttccgacattgccgtggaatgggagtccaatggccagcctgagaacaactacaagaccacacctcctgtgctggactccgacggctccttctttctgtactctcgcctgaccgtggacaagtctaggtggcaagagggcaacgtgttctcctgctctgtgctgcacgaggccctgcacaatcactacacccagaagtccctgtctctgtctcttggcggaggcggaggatctgctcctacctccagctccaccaagaaaacccagctccagttggagcatctgctgctggacctccagatgatcctgaatggcatcaacaattacaagaaccccaagctgaccgccatgctgaccgctaagttctacatgcccaagaaggccaccgagctgaagcacctccagtgcctggaagaggaactgaagcccctggaagaagtgctgaatctggcccagtccaagaacttccacctgaggcctagggacctgatctccaacatcaacgtgatcgtgctggaactgaaaggctccgagacaaccttcatgtgcgagtacgccgacgagacagccaccatcgtggaatttctgaaccggtggatcaccttctgccagtccatcatctccacactgacc

SEQ ID NO: 19 - protein, 367 aa, Artificial Sequence
  fusion protein (GI101C2)
AESKYGPPCPPCPAPEAAGGPSVFLFPPKPKDQLMISRTPEVTCVVVDVSQEDPEVQFNWYVDGVEVHNAKTKPREEQFNSTYRVVSVLTVLHQDWLNGKEYKCKVSNKGLPSSIEKTISKAKGQPREPQVYTLPPSQEEMTKNQVSLTCLVKGFYPSDIAVEWESNGQPENNYKTTPPVLDSDGSFFLYSRLTVDKSRWQEGNVFSCSVLHEALHNHYTQKSLSLSLGGGGGSAPTSSSTKKTQLQLEHLLLDLQMILNGINNYKNPKLTAMLTAKFYMPKKATELKHLQCLEEELKPLEEVLNLAQSKNFHLRPRDLISNINVIVLELKGSETTFMCEYADETATIVEFLNRWITFCQSIISTLT

SEQ ID NO: 20 - DNA, 1434 bp, Artificial Sequence
  nucleotiedes coding fusion protein (mGI101C1)
atggatgctatgctgagaggcctgtgttgcgtgctgctgctgtgtggcgctgtgttcgtgtctccttctcacgctgtggacgagcagctctccaagtccgtgaaggataaggtcctgctgccttgccggtacaactctcctcacgaggacgagtctgaggaccggatctactggcagaaacacgacaaggtggtgctgtccgtgatcgccggaaagctgaaagtgtggcctgagtacaagaacaggaccctgtacgacaacaccacctacagcctgatcatcctgggcctcgtgctgagcgatagaggcacctattcttgcgtggtgcagaagaaagagcggggcacctacgaagtgaagcacctggctctggtcaagctgtccatcaaggccgacttcagcacccctaacatcaccgagtctggcaacccttccgccgacaccaagagaatcacctgtttcgcctctggcggcttccctaagcctcggttctcttggctggaaaacggcagagagctgcccggcatcaataccaccatttctcaggacccagagtccgagctgtacaccatctccagccagctcgactttaacaccaccagaaaccacaccatcaagtgcctgattaagtacggcgacgcccacgtgtccgaggactttacttgggagaaacctcctgaggaccctcctgactctggatctggcggcggaggttctggcggaggtggaagcggaggcggaggatctgctgagtctaagtatggccctccttgtcctccatgtcctgctccagaagctgctggcggaccctctgtgttcctgtttcctccaaagcctaaggaccagctcatgatctctcggacccctgaagtgacctgcgtggtggtggatgtgtctcaagaggaccctgaggtgcagttcaattggtacgtggacggcgtggaagtgcacaacgccaagaccaagcctagagaggaacagttcaactccacctatagagtggtgtccgtgctgaccgtgctgcaccaggattggctgaacggcaaagagtacaagtgcaaggtgtccaacaagggcctgccttccagcatcgaaaagaccatcagcaaggctaagggccagcctagggaaccccaggtttacaccctgcctccaagccaagaggaaatgaccaagaaccaggtgtccctgacctgcctggtcaagggcttctacccttccgacattgccgtggaatgggagtccaatggccagcctgagaacaactacaagaccacacctcctgtgctggactccgacggctccttctttctgtactctcgcctgaccgtggacaagtctaggtggcaagagggcaacgtgttctcctgctctgtgctgcacgaggctctgcacaaccactacacccagaagtccctgtctctgtccctgggc

SEQ ID NO: 21 - protein, 478 aa, Artificial Sequence
  fusion protein (mGI101C1)
MDAMLRGLCCVLLLCGAVFVSPSHAVDEQLSKSVKDKVLLPCRYNSPHEDESEDRIYWQKHDKVVLSVIAGKLKVWPEYKNRTLYDNTTYSLIILGLVLSDRGTYSCVVQKKERGTYEVKHLALVKLSIKADFSTPNITESGNPSADTKRITCFASGGFPKPRFSWLENGRELPGINTTISQDPESELYTISSQLDFNTTRNHTIKCLIKYGDAHVSEDFTWEKPPEDPPDSGSGGGGSGGGGSGGGGSAESKYGPPCPPCPAPEAAGGPSVFLFPPKPKDQLMISRTPEVTCVVVDVSQEDPEVQFNWYVDGVEVHNAKTKPREEQFNSTYRVVSVLTVLHQDWLNGKEYKCKVSNKGLPSSIEKTISKAKGQPREPQVYTLPPSQEEMTKNQVSLTCLVKGFYPSDIAVEWESNGQPENNYKTTPPVLDSDGSFFLYSRLTVDKSRWQEGNVFSCSVLHEALHNHYTQKSLSLSLG

SEQ ID NO: 22 - protein, 133 aa, Artificial Sequence
  variants of IL-2 (3M, M45)
APTSSSTKKTQLQLEHLLLDLQMILNGINNYKNPKLTAMLTAKFAMPKKATELKHLQCLEEELKPLEEVLNLAQSKNFHLRPRDLISNINVIVLELKGSETTFMCEYADETATIVEFLNRWITFCQSIISTLT

SEQ ID NO: 23 - protein, 133 aa, Artificial Sequence
  variants of IL-2 (3M, M61)
APTSSSTKKTQLQLEHLLLDLQMILNGINNYKNPKLTAMLTAKFYMPKKATELKHLQCLERELKPLEEVLNLAQSKNFHLRPRDLISNINVIVLELKGSETTFMCEYADETATIVEFLNRWITFCQSIISTLT

SEQ ID NO: 24 - protein, 133 aa, Artificial Sequence
  variants of IL-2 (3M, M72)
APTSSSTKKTQLQLEHLLLDLQMILNGINNYKNPKLTAMLTAKFYMPKKATELKHLQCLEEELKPLEEVLNGAQSKNFHLRPRDLISNINVIVLELKGSETTFMCEYADETATIVEFLNRWITFCQSIISTLT

SEQ ID NO: 25 - DNA, 1851 bp, Artificial Sequence
  nucleotiedes coding fusion protein (GI102-M45)
atggatgctatgctgagaggcctgtgttgcgtgctgctgctgtgtggcgctgtgttcgtgtctccttctcacgctgtgatccacgtgaccaaagaagtgaaagaggtcgccacactgtcctgcggccacaacgtttcagtggaagaactggcccagaccaggatctactggcagaaagaaaagaaaatggtgctgaccatgatgtccggcgacatgaacatctggcctgagtacaagaaccggaccatcttcgacatcaccaacaacctgtccatcgtgattctggccctgaggccttctgatgagggcacctatgagtgcgtggtgctgaagtacgagaaggacgccttcaagcgcgagcacctggctgaagtgacactgtccgtgaaggccgactttcccacaccttccatctccgacttcgagatccctacctccaacatccggcggatcatctgttctacctctggcggctttcctgagcctcacctgtcttggctggaaaacggcgaggaactgaacgccatcaacaccaccgtgtctcaggaccccgaaaccgagctgtacgctgtgtcctccaagctggacttcaacatgaccaccaaccacagcttcatgtgcctgattaagtacggccacctgagagtgaaccagaccttcaactggaacaccaccaagcaagagcacttccctgacaatggatctggcggcggaggttctggcggaggtggaagcggaggcggaggatctgctgagtctaagtatggccctccttgtcctccatgtcctgctccagaagctgctggcggaccctctgtgttcctgtttcctccaaagcctaaggaccagctcatgatctctcggacacccgaagtgacctgcgtggtggtggatgtgtctcaagaggaccctgaggtgcagttcaattggtacgtggacggcgtggaagtgcacaacgccaagaccaagcctagagaggaacagttcaactccacctacagagtggtgtccgtgctgaccgtgctgcaccaggattggctgaacggcaaagagtacaagtgcaaggtgtccaacaagggcctgccttccagcatcgaaaagaccatctccaaggctaagggccagcctagggaaccccaggtttacaccctgcctccaagccaagaggaaatgaccaagaaccaggtgtccctgacctgcctggtcaagggcttctacccttccgacattgccgtggaatgggagtccaatggccagcctgagaacaactacaagaccacacctcctgtgctggactccgacggctccttctttctgtactctcgcctgaccgtggacaagtctagatggcaagagggcaacgtgttctcctgctctgtgctgcacgaggccctgcacaatcactacacccagaagtccctgtctctgtctcttggaggtggtggcggttctgcccctaccagctcctctaccaagaaaacccagctccagttggagcatctgctgctggacctccagatgattctgaacgggatcaacaactataagaaccccaagctgaccgccatgctgaccgctaagttcgccatgcccaagaaggccaccgagctgaagcacctccagtgcctggaagaagaactgaagcccctggaagaggtgctgaatctggcccagtccaagaacttccacctgaggccacgggacctgatcagcaacatcaacgtgatcgtgctggaactgaagggctccgagacaacctttatgtgcgagtacgccgacgagacagccaccatcgtggaatttctgaaccggtggatcaccttctgccagagcatcatctccacactgacc

SEQ ID NO: 26 - protein, 592 aa, Artificial Sequence
  fusion protein (GI102-M45)
VIHVTKEVKEVATLSCGHNVSVEELAQTRIYWQKEKKMVLTMMSGDMNIWPEYKNRTIFDITNNLSIVILALRPSDEGTYECVVLKYEKDAFKREHLAEVTLSVKADFPTPSISDFEIPTSNIRRIICSTSGGFPEPHLSWLENGEELNAINTTVSQDPETELYAVSSKLDFNMTTNHSFMCLIKYGHLRVNQTFNWNTTKQEHFPDNGSGGGGSGGGGSGGGGSAESKYGPPCPPCPAPEAAGGPSVFLFPPKPKDQLMISRTPEVTCVVVDVSQEDPEVQFNWYVDGVEVHNAKTKPREEQFNSTYRVVSVLTVLHQDWLNGKEYKCKVSNKGLPSSIEKTISKAKGQPREPQVYTLPPSQEEMTKNQVSLTCLVKGFYPSDIAVEWESNGQPENNYKTTPPVLDSDGSFFLYSRLTVDKSRWQEGNVFSCSVLHEALHNHYTQKSLSLSLGGGGGSAPTSSSTKKTQLQLEHLLLDLQMILNGINNYKNPKLTAMLTAKFAMPKKATELKHLQCLEEELKPLEEVLNLAQSKNFHLRPRDLISNINVIVLELKGSETTFMCEYADETATIVEFLNRWITFCQSIISTLT

SEQ ID NO: 27 - DNA, 1851 bp, Artificial Sequence
  nucleotiedes coding fusion protein (GI102-M61)
atggatgctatgctgagaggcctgtgttgcgtgctgctgctgtgtggcgctgtgttcgtgtctccttctcacgctgtgatccacgtgaccaaagaagtgaaagaggtcgccacactgtcctgcggccacaacgtttcagtggaagaactggcccagaccaggatctactggcagaaagaaaagaaaatggtgctgaccatgatgtccggcgacatgaacatctggcctgagtacaagaaccggaccatcttcgacatcaccaacaacctgtccatcgtgattctggccctgaggccttctgatgagggcacctatgagtgcgtggtgctgaagtacgagaaggacgccttcaagcgcgagcacctggctgaagtgacactgtccgtgaaggccgactttcccacaccttccatctccgacttcgagatccctacctccaacatccggcggatcatctgttctacctctggcggctttcctgagcctcacctgtcttggctggaaaacggcgaggaactgaacgccatcaacaccaccgtgtctcaggaccccgaaaccgagctgtacgctgtgtcctccaagctggacttcaacatgaccaccaaccacagcttcatgtgcctgattaagtacggccacctgagagtgaaccagaccttcaactggaacaccaccaagcaagagcacttccctgacaatggatctggcggcggaggttctggcggaggtggaagcggaggcggaggatctgctgagtctaagtatggccctccttgtcctccatgtcctgctccagaagctgctggcggaccctctgtgttcctgtttcctccaaagcctaaggaccagctcatgatctctcggacacccgaagtgacctgcgtggtggtggatgtgtctcaagaggaccctgaggtgcagttcaattggtacgtggacggcgtggaagtgcacaacgccaagaccaagcctagagaggaacagttcaactccacctacagagtggtgtccgtgctgaccgtgctgcaccaggattggctgaacggcaaagagtacaagtgcaaggtgtccaacaagggcctgccttccagcatcgaaaagaccatctccaaggctaagggccagcctagggaaccccaggtttacaccctgcctccaagccaagaggaaatgaccaagaaccaggtgtccctgacctgcctggtcaagggcttctacccttccgacattgccgtggaatgggagtccaatggccagcctgagaacaactacaagaccacacctcctgtgctggactccgacggctccttctttctgtactctcgcctgaccgtggacaagtctagatggcaagagggcaacgtgttctcctgctctgtgctgcacgaggccctgcacaatcactacacccagaagtccctgtctctgtctcttggaggtggtggcggttctgcccctaccagctcctctaccaagaaaacccagctccagttggagcatctgctgctggacctccagatgattctgaacgggatcaacaactataagaaccccaagctgaccgccatgctgaccgctaagttctacatgcccaagaaggccaccgagctgaagcacctccagtgcctggaaagggaactgaagcccctggaagaggtgctgaatctggcccagtccaagaacttccacctgaggccacgggacctgatcagcaacatcaacgtgatcgtgctggaactgaagggctccgagacaacctttatgtgcgagtacgccgacgagacagccaccatcgtggaatttctgaaccggtggatcaccttctgccagagcatcatctccacactgacc

SEQ ID NO: 28 - protein, 592 aa, Artificial Sequence
  fusion protein (GI102-M61)
VIHVTKEVKEVATLSCGHNVSVEELAQTRIYWQKEKKMVLTMMSGDMNIWPEYKNRTIFDITNNLSIVILALRPSDEGTYECVVLKYEKDAFKREHLAEVTLSVKADFPTPSISDFEIPTSNIRRIICSTSGGFPEPHLSWLENGEELNAINTTVSQDPETELYAVSSKLDFNMTTNHSFMCLIKYGHLRVNQTFNWNTTKQEHFPDNGSGGGGSGGGGSGGGGSAESKYGPPCPPCPAPEAAGGPSVFLFPPKPKDQLMISRTPEVTCVVVDVSQEDPEVQFNWYVDGVEVHNAKTKPREEQFNSTYRVVSVLTVLHQDWLNGKEYKCKVSNKGLPSSIEKTISKAKGQPREPQVYTLPPSQEEMTKNQVSLTCLVKGFYPSDIAVEWESNGQPENNYKTTPPVLDSDGSFFLYSRLTVDKSRWQEGNVFSCSVLHEALHNHYTQKSLSLSLGGGGGSAPTSSSTKKTQLQLEHLLLDLQMILNGINNYKNPKLTAMLTAKFYMPKKATELKHLQCLERELKPLEEVLNLAQSKNFHLRPRDLISNINVIVLELKGSETTFMCEYADETATIVEFLNRWITFCQSIISTLT

SEQ ID NO: 29 - DNA, 1857 bp, Artificial Sequence
  nucleotiedes coding fusion protein (GI102-M72)
atggatgctatgctgagaggcctgtgttgcgtgctgctgctgtgtggcgctgtgttcgtgtctccttctcacgctgtgatccacgtgaccaaagaagtgaaagaggtcgccacactgtcctgcggccacaacgtttcagtggaagaactggcccagaccaggatctactggcagaaagaaaagaaaatggtgctgaccatgatgtccggcgacatgaacatctggcctgagtacaagaaccggaccatcttcgacatcaccaacaacctgtccatcgtgattctggccctgaggccttctgatgagggcacctatgagtgcgtggtgctgaagtacgagaaggacgccttcaagcgcgagcacctggctgaagtgacactgtccgtgaaggccgactttcccacaccttccatctccgacttcgagatccctacctccaacatccggcggatcatctgttctacctctggcggctttcctgagcctcacctgtcttggctggaaaacggcgaggaactgaacgccatcaacaccaccgtgtctcaggaccccgaaaccgagctgtacgctgtgtcctccaagctggacttcaacatgaccaccaaccacagcttcatgtgcctgattaagtacggccacctgagagtgaaccagaccttcaactggaacaccaccaagcaagagcacttccctgacaatggatctggcggcggaggttctggcggaggtggaagcggaggcggaggatctgctgagtctaagtatggccctccttgtcctccatgtcctgctccagaagctgctggcggaccctctgtgttcctgtttcctccaaagcctaaggaccagctcatgatctctcggacacccgaagtgacctgcgtggtggtggatgtgtctcaagaggaccctgaggtgcagttcaattggtacgtggacggcgtggaagtgcacaacgccaagaccaagcctagagaggaacagttcaactccacctacagagtggtgtccgtgctgaccgtgctgcaccaggattggctgaacggcaaagagtacaagtgcaaggtgtccaacaagggcctgccttccagcatcgaaaagaccatctccaaggctaagggccagcctagggaaccccaggtttacaccctgcctccaagccaagaggaaatgaccaagaaccaggtgtccctgacctgcctggtcaagggcttctacccttccgacattgccgtggaatgggagtccaatggccagcctgagaacaactacaagaccacacctcctgtgctggactccgacggctccttctttctgtactctcgcctgaccgtggacaagtctagatggcaagagggcaacgtgttctcctgctctgtgctgcacgaggccctgcacaatcactacacccagaagtccctgtctctgtctcttggaggtggtggcggttctgcccctaccagctcctctaccaagaaaacccagctccagttggagcatctgctgctggacctccagatgattctgaacgggatcaacaactataagaaccccaagctgaccgccatgctgaccgctaagttctacatgcccaagaaggccaccgagctgaagcacctccagtgcctggaagaagaactgaagcccctggaagaggtgctgaatggggcccagtccaagaacttccacctgaggccacgggacctgatcagcaacatcaacgtgatcgtgctggaactgaagggctccgagacaacctttatgtgcgagtacgccgacgagacagccaccatcgtggaatttctgaaccggtggatcaccttctgccagagcatcatctccacactgacctgatga

SEQ ID NO: 30 - protein, 592 aa, Artificial Sequence
  fusion protein (GI102-M72)
VIHVTKEVKEVATLSCGHNVSVEELAQTRIYWQKEKKMVLTMMSGDMNIWPEYKNRTIFDITNNLSIVILALRPSDEGTYECVVLKYEKDAFKREHLAEVTLSVKADFPTPSISDFEIPTSNIRRIICSTSGGFPEPHLSWLENGEELNAINTTVSQDPETELYAVSSKLDFNMTTNHSFMCLIKYGHLRVNQTFNWNTTKQEHFPDNGSGGGGSGGGGSGGGGSAESKYGPPCPPCPAPEAAGGPSVFLFPPKPKDQLMISRTPEVTCVVVDVSQEDPEVQFNWYVDGVEVHNAKTKPREEQFNSTYRVVSVLTVLHQDWLNGKEYKCKVSNKGLPSSIEKTISKAKGQPREPQVYTLPPSQEEMTKNQVSLTCLVKGFYPSDIAVEWESNGQPENNYKTTPPVLDSDGSFFLYSRLTVDKSRWQEGNVFSCSVLHEALHNHYTQKSLSLSLGGGGGSAPTSSSTKKTQLQLEHLLLDLQMILNGINNYKNPKLTAMLTAKFYMPKKATELKHLQCLEEELKPLEEVLNGAQSKNFHLRPRDLISNINVIVLELKGSETTFMCEYADETATIVEFLNRWITFCQSIISTLT

SEQ ID NO: 31 - DNA, 1851 bp, Artificial Sequence
  nucleotiedes coding fusion protein (GI101w)
atggatgctatgctgagaggcctgtgttgcgtgctgctgctgtgtggcgctgtgttcgtgtctccttctcacgctgtgatccacgtgaccaaagaagtgaaagaggtcgccacactgtcctgcggccacaacgtttcagtggaagaactggcccagaccaggatctactggcagaaagaaaagaaaatggtgctgaccatgatgtccggcgacatgaacatctggcctgagtacaagaaccggaccatcttcgacatcaccaacaacctgtccatcgtgattctggccctgaggccttctgatgagggcacctatgagtgcgtggtgctgaagtacgagaaggacgccttcaagcgcgagcacctggctgaagtgacactgtccgtgaaggccgactttcccacaccttccatctccgacttcgagatccctacctccaacatccggcggatcatctgttctacctctggcggctttcctgagcctcacctgtcttggctggaaaacggcgaggaactgaacgccatcaacaccaccgtgtctcaggaccccgaaaccgagctgtacgctgtgtcctccaagctggacttcaacatgaccaccaaccacagcttcatgtgcctgattaagtacggccacctgagagtgaaccagaccttcaactggaacaccaccaagcaagagcacttccctgacaatggatctggcggcggaggttctggcggaggtggaagcggaggcggaggatctgctgagtctaagtatggccctccttgtcctccatgtcctgctccagaagctgctggcggaccctctgtgttcctgtttcctccaaagcctaaggaccagctcatgatctctcggacacccgaagtgacctgcgtggtggtggatgtgtctcaagaggaccctgaggtgcagttcaattggtacgtggacggcgtggaagtgcacaacgccaagaccaagcctagagaggaacagttcaactccacctacagagtggtgtccgtgctgaccgtgctgcaccaggattggctgaacggcaaagagtacaagtgcaaggtgtccaacaagggcctgccttccagcatcgaaaagaccatctccaaggctaagggccagcctagggaaccccaggtttacaccctgcctccaagccaagaggaaatgaccaagaaccaggtgtccctgacctgcctggtcaagggcttctacccttccgacattgccgtggaatgggagtccaatggccagcctgagaacaactacaagaccacacctcctgtgctggactccgacggctccttctttctgtactctcgcctgaccgtggacaagtctagatggcaagagggcaacgtgttctcctgctctgtgctgcacgaggccctgcacaatcactacacccagaagtccctgtctctgtctcttggaggtggtggcggttctgcccctaccagctcctctaccaagaaaacccagctccagttggagcatctgctgctggacctccagatgattctgaacgggatcaacaactataagaaccccaagctgacccgcatgctgacctttaagttctacatgcccaagaaggccaccgagctgaagcacctccagtgcctggaagaagaactgaagcccctggaagaggtgctgaatctggcccagtccaagaacttccacctgaggccacgggacctgatcagcaacatcaacgtgatcgtgctggaactgaagggctccgagacaacctttatgtgcgagtacgccgacgagacagccaccatcgtggaatttctgaaccggtggatcaccttctgccagagcatcatctccacactgacc

SEQ ID NO: 32 - protein, 592 aa, Artificial Sequence
  fusion protein (GI101w)
VIHVTKEVKEVATLSCGHNVSVEELAQTRIYWQKEKKMVLTMMSGDMNIWPEYKNRTIFDITNNLSIVILALRPSDEGTYECVVLKYEKDAFKREHLAEVTLSVKADFPTPSISDFEIPTSNIRRIICSTSGGFPEPHLSWLENGEELNAINTTVSQDPETELYAVSSKLDFNMTTNHSFMCLIKYGHLRVNQTFNWNTTKQEHFPDNGSGGGGSGGGGSGGGGSAESKYGPPCPPCPAPEAAGGPSVFLFPPKPKDQLMISRTPEVTCVVVDVSQEDPEVQFNWYVDGVEVHNAKTKPREEQFNSTYRVVSVLTVLHQDWLNGKEYKCKVSNKGLPSSIEKTISKAKGQPREPQVYTLPPSQEEMTKNQVSLTCLVKGFYPSDIAVEWESNGQPENNYKTTPPVLDSDGSFFLYSRLTVDKSRWQEGNVFSCSVLHEALHNHYTQKSLSLSLGGGGGSAPTSSSTKKTQLQLEHLLLDLQMILNGINNYKNPKLTRMLTFKFYMPKKATELKHLQCLEEELKPLEEVLNLAQSKNFHLRPRDLISNINVIVLELKGSETTFMCEYADETATIVEFLNRWITFCQSIISTLT

SEQ ID NO: 33 - DNA, 1848 bp, Artificial Sequence
  nucleotiedes coding fusion protein (mGI102-M61)
atggatgctatgctgagaggcctgtgttgcgtgctgctgctgtgtggcgctgtgttcgtgtctccttctcacgctgtggacgagcagctctccaagtccgtgaaggataaggtcctgctgccttgccggtacaactctcctcacgaggacgagtctgaggaccggatctactggcagaaacacgacaaggtggtgctgtccgtgatcgccggaaagctgaaagtgtggcctgagtacaagaacaggaccctgtacgacaacaccacctacagcctgatcatcctgggcctcgtgctgagcgatagaggcacctattcttgcgtggtgcagaagaaagagcggggcacctacgaagtgaagcacctggctctggtcaagctgtccatcaaggccgacttcagcacccctaacatcaccgagtctggcaacccttccgccgacaccaagagaatcacctgtttcgcctctggcggcttccctaagcctcggttctcttggctggaaaacggcagagagctgcccggcatcaataccaccatttctcaggacccagagtccgagctgtacaccatctccagccagctcgactttaacaccaccagaaaccacaccatcaagtgcctgattaagtacggcgacgcccacgtgtccgaggactttacttgggagaaacctcctgaggaccctcctgactctggatctggcggcggaggttctggcggaggtggaagcggaggcggaggatctgctgagtctaagtatggccctccttgtcctccatgtcctgctccagaagctgctggcggaccctctgtgttcctgtttcctccaaagcctaaggaccagctcatgatctctcggacccctgaagtgacctgcgtggtggtggatgtgtctcaagaggaccctgaggtgcagttcaattggtacgtggacggcgtggaagtgcacaacgccaagaccaagcctagagaggaacagttcaactccacctatagagtggtgtccgtgctgaccgtgctgcaccaggattggctgaacggcaaagagtacaagtgcaaggtgtccaacaagggcctgccttccagcatcgaaaagaccatcagcaaggctaagggccagcctagggaaccccaggtttacaccctgcctccaagccaagaggaaatgaccaagaaccaggtgtccctgacctgcctggtcaagggcttctacccttccgacattgccgtggaatgggagtccaatggccagcctgagaacaactacaagaccacacctcctgtgctggactccgacggctccttctttctgtactctcgcctgaccgtggacaagtctaggtggcaagagggcaacgtgttctcctgctctgtgctgcacgaggctctgcacaaccactacacccagaagtccctgtctctgtctcttggaggtggtggcggttctgcccctacctccagctctaccaagaaaacccagctccagttggagcatctgctgctggacctccagatgatcctgaatggcatcaacaattacaagaaccccaagctgaccgccatgctgaccgctaagttctacatgcccaagaaggccaccgagctgaagcacttgcagtgcctggaaagggaactgaagcccctggaagaagtgctgaatctggcccagtccaagaacttccacctgaggcctagggacctgatctccaacatcaacgtgatcgtgctggaactgaaaggctccgagacaaccttcatgtgcgagtacgccgacgagacagccaccatcgtggaatttctgaaccggtggatcaccttctgccagagcatcatctccacactgacc

SEQ ID NO: 34 - protein, 616 aa, Artificial Sequence
  fusion protein (mGI102-M61)
MDAMLRGLCCVLLLCGAVFVSPSHAVDEQLSKSVKDKVLLPCRYNSPHEDESEDRIYWQKHDKVVLSVIAGKLKVWPEYKNRTLYDNTTYSLIILGLVLSDRGTYSCVVQKKERGTYEVKHLALVKLSIKADFSTPNITESGNPSADTKRITCFASGGFPKPRFSWLENGRELPGINTTISQDPESELYTISSQLDFNTTRNHTIKCLIKYGDAHVSEDFTWEKPPEDPPDSGSGGGGSGGGGSGGGGSAESKYGPPCPPCPAPEAAGGPSVFLFPPKPKDQLMISRTPEVTCVVVDVSQEDPEVQFNWYVDGVEVHNAKTKPREEQFNSTYRVVSVLTVLHQDWLNGKEYKCKVSNKGLPSSIEKTISKAKGQPREPQVYTLPPSQEEMTKNQVSLTCLVKGFYPSDIAVEWESNGQPENNYKTTPPVLDSDGSFFLYSRLTVDKSRWQEGNVFSCSVLHEALHNHYTQKSLSLSLGGGGGSAPTSSSTKKTQLQLEHLLLDLQMILNGINNYKNPKLTAMLTAKFYMPKKATELKHLQCLERELKPLEEVLNLAQSKNFHLRPRDLISNINVIVLELKGSETTFMCEYADETATIVEFLNRWITFCQSIISTLT

SEQ ID NO: 35 - protein, 153 aa, Artificial Sequence
  wild type hIL-2
MYRMQLLSCIALSLALVTNSAPTSSSTKKTQLQLEHLLLDLQMILNGINNYKNPKLTRMLTFKFYMPKKATELKHLQCLEEELKPLEEVLNLAQSKNFHLRPRDLISNINVIVLELKGSETTFMCEYADETATIVEFLNRWITFCQSIISTLT

SEQ ID NO: 36 - protein, 158 aa, Artificial Sequence
  IL-2 with signal sequence
MDAMLRGLCCVLLLCGAVFVSPSHAAPTSSSTKKTQLQLEHLLLDLQMILNGINNYKNPKLTRMLTFKFYMPKKATELKHLQCLEEELKPLEEVLNLAQSKNFHLRPRDLISNINVIVLELKGSETTFMCEYADETATIVEFLNRWITFCQSIISTLT

SEQ ID NO: 37 - DNA, 474 bp, Artificial Sequence
  nucleotide sequence coding IL-2 with signal sequence
atggatgctatgctgagaggcctgtgttgcgtgctgctgctgtgtggcgctgtgttcgtgtctccttctcacgctgcccctaccagctcctctaccaagaaaacccagctccagttggagcatctgctgctggacctccagatgattctgaacgggatcaacaactataagaaccccaagctgacccgcatgctgacctttaagttctacatgcccaagaaggccaccgagctgaagcacctccagtgcctggaagaagaactgaagcccctggaagaggtgctgaatctggcccagtccaagaacttccacctgaggccacgggacctgatcagcaacatcaacgtgatcgtgctggaactgaagggctccgagacaacctttatgtgcgagtacgccgacgagacagccaccatcgtggaatttctgaaccggtggatcaccttctgccagagcatcatctccacactgacc

SEQ ID NO: 38 - protein, 13 aa, Artificial Sequence
  hinge
AESKYGPPCPPCP

SEQ ID NO: 39 - DNA, 1461 bp, Artificial Sequence
  nucleotides coding CD80-Fc protein
ggatccgccaccatggatgctatgctgagaggcctgtgttgcgtgctgctgctgtgtggcgctgtgttcgtgtctccttctcacgctgtgatccacgtgaccaaagaagtgaaagaggtcgccacactgtcctgcggccacaacgtttcagtggaagaactggcccagaccaggatctactggcagaaagaaaagaaaatggtgctgaccatgatgtccggcgacatgaacatctggcctgagtacaagaaccggaccatcttcgacatcaccaacaacctgtccatcgtgattctggccctgaggccttctgatgagggcacctatgagtgcgtggtgctgaagtacgagaaggacgccttcaagcgcgagcacctggctgaagtgacactgtccgtgaaggccgactttcccacaccttccatctccgacttcgagatccctacctccaacatccggcggatcatctgttctacctctggcggctttcctgagcctcacctgtcttggctggaaaacggcgaggaactgaacgccatcaacaccaccgtgtctcaggaccccgaaaccgagctgtacgctgtgtcctccaagctggacttcaacatgaccaccaaccacagcttcatgtgcctgattaagtacggccacctgagagtgaaccagaccttcaactggaacaccaccaagcaagagcacttccctgacaatggatctggcggcggaggttctggcggaggtggaagcggaggcggaggatctgctgagtctaagtatggccctccttgtcctccatgtcctgctccagaagctgctggcggaccctctgtgttcctgtttcctccaaagcctaaggaccagctcatgatctctcggacacccgaagtgacctgcgtggtggtggatgtgtctcaagaggaccctgaggtgcagttcaattggtacgtggacggcgtggaagtgcacaacgccaagaccaagcctagagaggaacagttcaactccacctacagagtggtgtccgtgctgaccgtgctgcaccaggattggctgaacggcaaagagtacaagtgcaaggtgtccaacaagggcctgccttccagcatcgaaaagaccatctccaaggctaagggccagcctagggaaccccaggtttacaccctgcctccaagccaagaggaaatgaccaagaaccaggtgtccctgacctgcctggtcaagggcttctacccttccgacattgccgtggaatgggagtccaatggccagcctgagaacaactacaagaccacacctcctgtgctggactccgacggctccttctttctgtactctcgcctgaccgtggacaagtctaggtggcaagagggcaacgtgttctcctgctctgtgctgcacgaggccctgcacaatcactacacccagaagtccctgtctctgtccctgggctgatgactcgag

SEQ ID NO: 40 - protein, 479 aa, Artificial Sequence
  CD80-Fc protein
MDAMLRGLCCVLLLCGAVFVSPSHAVIHVTKEVKEVATLSCGHNVSVEELAQTRIYWQKEKKMVLTMMSGDMNIWPEYKNRTIFDITNNLSIVILALRPSDEGTYECVVLKYEKDAFKREHLAEVTLSVKADFPTPSISDFEIPTSNIRRIICSTSGGFPEPHLSWLENGEELNAINTTVSQDPETELYAVSSKLDFNMTTNHSFMCLIKYGHLRVNQTFNWNTTKQEHFPDNGSGGGGSGGGGSGGGGSAESKYGPPCPPCPAPEAAGGPSVFLFPPKPKDQLMISRTPEVTCVVVDVSQEDPEVQFNWYVDGVEVHNAKTKPREEQFNSTYRVVSVLTVLHQDWLNGKEYKCKVSNKGLPSSIEKTISKAKGQPREPQVYTLPPSQEEMTKNQVSLTCLVKGFYPSDIAVEWESNGQPENNYKTTPPVLDSDGSFFLYSRLTVDKSRWQEGNVFSCSVLHEALHNHYTQKSLSLSLG

SEQ ID NO: 41 - DNA, 1851 bp, Artificial Sequence; identical to SEQ ID NO: 31
  nucleotiedes coding fusion protein (hCD80-Fc-IL2wt)

SEQ ID NO: 42 - protein, 367 aa, Artificial Sequence
  Fc-IL2wt
AESKYGPPCPPCPAPEAAGGPSVFLFPPKPKDQLMISRTPEVTCVVVDVSQEDPEVQFNWYVDGVEVHNAKTKPREEQFNSTYRVVSVLTVLHQDWLNGKEYKCKVSNKGLPSSIEKTISKAKGQPREPQVYTLPPSQEEMTKNQVSLTCLVKGFYPSDIAVEWESNGQPENNYKTTPPVLDSDGSFFLYSRLTVDKSRWQEGNVFSCSVLHEALHNHYTQKSLSLSLGGGGGSAPTSSSTKKTQLQLEHLLLDLQMILNGINNYKNPKLTRMLTFKFYMPKKATELKHLQCLEEELKPLEEVLNLAQSKNFHLRPRDLISNINVIVLELKGSETTFMCEYADETATIVEFLNRWITFCQSIISTLT

SEQ ID NO: 43 - DNA, 1176 bp, Artificial Sequence
  Fc-IL2wt
atggatgctatgctgagaggcctgtgttgcgtgctgctgctgtgtggcgctgtgttcgtgtctccttctcacgctgctgagtctaagtatggccctccttgtcctccatgtcctgctccagaagctgctggcggaccctctgtgttcctgtttcctccaaagcctaaggaccagctcatgatctctcggacacccgaagtgacctgcgtggtggtggatgtgtctcaagaggaccctgaggtgcagttcaattggtacgtggacggcgtggaagtgcacaacgccaagaccaagcctagagaggaacagttcaactccacctacagagtggtgtccgtgctgaccgtgctgcaccaggattggctgaacggcaaagagtacaagtgcaaggtgtccaacaagggcctgccttccagcatcgaaaagaccatctccaaggctaagggccagcctagggaaccccaggtttacaccctgcctccaagccaagaggaaatgaccaagaaccaggtgtccctgacctgcctggtcaagggcttctacccttccgacattgccgtggaatgggagtccaatggccagcctgagaacaactacaagaccacacctcctgtgctggactccgacggctccttctttctgtactctcgcctgaccgtggacaagtctagatggcaagagggcaacgtgttctcctgctctgtgctgcacgaggccctgcacaatcactacacccagaagtccctgtctctgtctcttggaggtggtggcggttctgcccctaccagctcctctaccaagaaaacccagctccagttggagcatctgctgctggacctccagatgattctgaacgggatcaacaactataagaaccccaagctgacccgcatgctgacctttaagttctacatgcccaagaaggccaccgagctgaagcacctccagtgcctggaagaagaactgaagcccctggaagaggtgctgaatctggcccagtccaagaacttccacctgaggccacgggacctgatcagcaacatcaacgtgatcgtgctggaactgaagggctccgagacaacctttatgtgcgagtacgccgacgagacagccaccatcgtggaatttctgaaccggtggatcaccttctgccagagcatcatctccacactgacc

SEQ ID NO: 44 - protein, 392 aa, Artificial Sequence
  Fc-IL2v2
MDAMLRGLCCVLLLCGAVFVSPSHAAESKYGPPCPPCPAPEAAGGPSVFLFPPKPKDQLMISRTPEVTCVVVDVSQEDPEVQFNWYVDGVEVHNAKTKPREEQFNSTYRVVSVLTVLHQDWLNGKEYKCKVSNKGLPSSIEKTISKAKGQPREPQVYTLPPSQEEMTKNQVSLTCLVKGFYPSDIAVEWESNGQPENNYKTTPPVLDSDGSFFLYSRLTVDKSRWQEGNVFSCSVLHEALHNHYTQKSLSLSLGGGGGSAPTSSSTKKTQLQLEHLLLDLQMILNGINNYKNPKLTAMLTAKFYMPKKATELKHLQCLEEELKPLEEVLNLAQSKNFHLRPRDLISNINVIVLELKGSETTFMCEYADETATIVEFLNRWITFCQSIISTLT

SEQ ID NO: 45 - DNA, 1200 bp, Artificial Sequence
  nucleotides coding Fc-IL2v2
ggatccgccaccatggatgctatgctgagaggcctgtgttgcgtgctgctgctgtgtggcgctgtgttcgtgtctccatctcacgccgctgagtctaagtacggccctccttgtcctccatgtcctgctccagaagctgctggcggaccctctgtgttcctgtttcctccaaagcctaaggaccagctcatgatctctcggacccctgaagtgacctgcgtggtggtggatgtgtctcaagaggaccctgaggtgcagttcaattggtacgtggacggcgtggaagtgcacaacgccaagaccaagcctagagaggaacagttcaactccacctacagagtggtgtccgtgctgaccgtgctgcaccaggattggctgaacggcaaagagtacaagtgcaaggtgtccaacaagggcctgccttccagcatcgaaaagaccatctccaaggctaagggccagcctagggaaccccaggtttacaccctgcctccaagccaagaggaaatgaccaagaaccaggtgtccctgacctgcctggtcaagggcttctacccttccgacattgccgtggaatgggagtccaatggccagcctgagaacaactacaagaccacacctcctgtgctggactccgacggctccttctttctgtactctcgcctgaccgtggacaagtctaggtggcaagagggcaacgtgttctcctgctctgtgctgcacgaggccctgcacaatcactacacccagaagtccctgtctctgtctcttggcggaggcggaggatctgctcctacctccagctccaccaagaaaacccagctccagttggagcatctgctgctggacctccagatgatcctgaatggcatcaacaattacaagaaccccaagctgaccgccatgctgaccgctaagttctacatgcccaagaaggccaccgagctgaagcacctccagtgcctggaagaggaactgaagcccctggaagaagtgctgaatctggcccagtccaagaacttccacctgaggcctagggacctgatctccaacatcaacgtgatcgtgctggaactgaaaggctccgagacaaccttcatgtgcgagtacgccgacgagacagccaccatcgtggaatttctgaaccggtggatcaccttctgccagtccatcatctccacactgacctgatgactcgag

SEQ ID NO: 46 - protein, 592 aa, Artificial Sequence; identical to SEQ ID NO: 32
  CD80-Fc-IL2wt